European Patent Specification EP 3 818 138 B1, published May 14, 2025. Title: Cleaning compositions and uses thereof. Applicant: Novozymes A/S. The sequence listing filed with the application follows.

SEQUENCE LISTING (43 sequences)

SEQ ID NO: 1 - protein, 359 aa, Aggregatibacter actinomycetemcomitans
CVKGNSIHPQKTSTKQTGLMLDIARHFYSPEVIKSFIDTISLSGGNFLHLHFSDHENYAIESHLLNQRAENAVQGKDGIYINPYTGKPFLSYRQLDDIKAYAKAKGIELIPELDSPNHMTAIFKLVQKDRGIKYLQGLKSRQVDDEIDITNADSIAFMQSLMSEVIDIFGDTSQHFHIGGDEFGYSVESNHEFITYANKLSYFLEKKGLKTRMWNDGLIKSTFEQINPNIEITYWSYDGDTQDKNEAAERRDMRVSLPELLAKGFTVLNYNSYYLYIVPKASPTFSQDAAFAAKDVIKNWDLGVWDGRNTKNRVQNTHEIAGAALSIWGEDAKALKDETIQKNTKSLLEAVIHKANGDE

SEQ ID NO: 2 - protein, 346 aa, Haemophilus sputorum
QNSTKQSGLMLDISRRFYSVETIKQFIDDIAQANGTFLHLHFADHENYALESTFLNQRAENAIVQNGIYINPKTNKPFLTYEQIDQIIRYAQEKQIELIPEVDSPAHIKGILTLLRLEKGEDYVNQIALNQDELNLDSPESLTMMKTLVDEVCYIFGYSAQHFHIGGDEFNYASNFIRYVNALNQHINQKGLITRMWNDGLLQQNIDELDKNIEITYWSFDGDAQEKNDIVERRATRISLPTLLDKGFKALNYNSYYLYFIPKDNGNIATDAKFALNDLKQNWQLLRWDGNYETQPIQQAENLIGAAFSIWGEHAGKLSDDVIHQATSPLIQATIIQTNAKTTGPN

SEQ ID NO: 3 - protein, 352 aa, Actinobacillus suis
MNHSQIKEAGLTLDIARRFYPVETIKQFIDTIHHAGGTFLHLHFSDHENYALESTYLDQSEANAIVKDGTYYNPKTNKPFLTYKQIHDIIYYAKSKNIELVPEVDTPNHMTAIFRLLEAKHGKDYVKKLKSKMNDEEIDITNPESIEVIKTLIAEVIYIFGHASEHFHIGGDEFGYSVETNHEFISYVNTLNQFINEKGKITRIWNDGLIKNNLNQLNKNVEITYWSYDGDAQESQDIAERRKIRANLPELLENGFKVLNYNSYYLYFVPKGNANITHDSKYATEDVLNNWKLGLWDGQNKENMVENTKNIIGSSLSIWGERSGSLSSEVIEESTQDLLKAVIQKTNDPKSH

SEQ ID NO: 4 - protein, 352 aa, Actinobacillus capsulatus DSM 19761
MNHSQIKEAGLTLDIARRFYPVETIKQFIDTIHHAGGTFLHLHFSDHENYALESTYLDQLEANAIVKDGTYYNPTTNKPFLTYKQINDIIYYAKSKNIELVPEVDTPNHMTAIFRLLEAKHSKDYVKRLKSKMNDEEIDITNLESIEVIKTLIAEVIYIFGHASEHFHIGGDEFGYSVETNHEFITYVNTLNQFINNKGKITRIWNDGLIKNNLNQLNKNVEITYWSYDGDAQESQDIAERRKIRVNLPELLENGFKVLNYNSYYLYFVPKGNANITHDSKHATEDVLKNWKLGLWDGQNKENIVENTKNIIGSSLSIWGEHSGSLSSAVIEESTQELLKAVIQKTNDPKSH

SEQ ID NO: 5 - protein, 352 aa, Actinobacillus equuli subsp. equuli
MNHSQIKEAGLTLDIARRFYPVETIKQFIDTIHHAGGTFLHLHFSDHENYALESSYLDQSEENAIVKDGTYYNPKTNKPFLTYKQIDDIIYYAKSKNIELVPEVDTPNHMTAIFNLLEIKHGEAYVKNLKSKMNDEEIDITNPESIEVIKTLIAEVIYIFGHASEHFHIGGDEFGYSVETNHEFISYVNTLNQFINEKGKITRIWNDGLIKNNLNQLNKNVEITYWSYDGDAQKSQDIAERRKIRADLPELLENGFKVLNYNSYYLYFVPKGNANITHDSKYATEDVLNNWKLGLWDGKNKENEVKNTKNIIGSSLSIWGERSGSLSSEVIEESTQDLLKAVIQKTNDPKSH

SEQ ID NO: 6 - protein, 359 aa, Aggregatibacter actinomycetemcomitans
CVKGNSIYPQKISTKQTGLMLDIARHFYSPEVIKSFIDTISLSGGNFLHLHFSDHENYAIESHLLNQRAENAVQGKDGIYINPYTGKPFLSYRQLDDIKAYAKAKGIELIPELDSPNHMTAIFKLVQKDRGVKYLQGLKSRQVDDEIDITNADSIAFMQSLMNEVIDIFGDTSQHFHIGGDEFGYSVESNHEFITYANKLSYFLEKKGLKTRMWNDGLIKSTFEQINPNIEITYWSYDGDTQDKNEAAERRDMRVSLPELLAKGFTVLNYNSYYLYIVPKASPTFSQDAAFAAKDVIKNWDLGVWDGRNTKNRVQNTHEIAGAALSIWGEDAKALKDETIQKNTKSLLEAVIHKTNGDE

SEQ ID NO: 7 - protein, 359 aa, Aggregatibacter actinomycetemcomitans
CVKGNSIYPQKTSTKQTGLMLDIARHFYSPEVIKSFIDTISLSGGNFLHLHFSDHENYAIESHLLNQRAENAVQGKDGIYINPYTGKPFLSYRQLDDIKAYAKAKGIELIPELDSPNHMTAIFKLVQKDRGVKYLQGLKSRQVDDEIDITNADSITFMQSLMSEVIDIFGDTSQHFHIGGDEFGYSVESNHEFITYANKLSYFLEKKGLKTRMWNDGLIKNTFEQINPNIEITYWSYDGDTQDKNEAAERRDMRVSLPELLAKGFTVLNYNSYYLYIVPKASPTFSQDAAFAAKDVIKNWDLGVWDGRNTKNRVQNTHEIAGAALSIWGEDAKALKDETIQKNTKSLLEAVIHKTNGDE

SEQ ID NO: 8 - protein, 351 aa, Actinobacillus pleuropneumoniae
MDLPKKESGLTLDIARRFYTVDTIKQFIDTIHQAGGTFLHLHFSDHENYALESSYLEQREENATEKNGTYFNPKTNKPFLTYKQLNEIIYYAKERNIEIVPEVDSPNHMTAIFDLLTLKHGKEYVKGLKSPYIAEEIDINNPEAVEVIKTLIGEVIYIFGHSSRHFHIGGDEFSYAVENNHEFIRYVNTLNDFINSKGLITRVWNDGLIKNNLSELNKNIEITYWSYDGDAQAKEDIQYRREIRADLPELLANGFKVLNYNSYYLYFVPKSGSNIHNDGKYAAEDVLNNWTLGKWDGKNSSNHVQNTQNIIGSSLSIWGERSSALNEQTIQQASKNLLKAVIQKTNDPKSH

SEQ ID NO: 9 - protein, 461 aa, Curtobacterium oceanosedimentum
ADRNTSAAEAAVTSIAPRATITGVAAISAATSSRTTVRTTLTLENRSGERESAADAWLYLAGGGARYALGHAPVRALAAGARATVRTTLRVPSRAPAGKYAVLACAGPYSKQACRTSGTTVTVGTAARARPETGVMLDVARAYYPVSLIEQYVDLLAEHGGGFLHLHLTDDQNVGIESAVLGQTPANAVLRNGVYTSRVTGRPFLSAAQARAISAYAAKRGIAIVPEVDSPGHMAAAFALLEARHGATWVDRIRSGESELDTSVPESATLAAELLREVTQTFPSSRTVHIGGDEWGADVSADERVGWMNAMAAAIGDREVWAWNDGIDRASVGRLDPRIHVTYWSFDGDTEDAAERRERRARRASATDLQRAGIDLLNYNSYYLYEVPTDLDPADSEYTVADLREHWSLRAWDGDSGARLAAPMSGAAVAIWGEDLDGAPSEALLRWSAPHVTAMIETAAS

SEQ ID NO: 10 - protein, 445 aa, Curtobacterium flaccumfaciens
DTAVSAVTVTKVTASTTGTVVRTTLKVENTAPVRKPASSVWLYLSAGTEKYTLGRVAVKALAAGSSTSVTAVRGTPSRAAAGKYSVLACAGAYSAKQCRTSTATVTTKPTKRARPETGVMLDVARAYYPVALIKRYIDLLADDGGRFLHLHLTDDQNVGIESTVLGQTPANADLDHGVYTSRVTHRPFLSAAQARTISAYGAERGVAIVPEIDTPGHMAAAFALLEAQHGTKWVDRIRSGENELDTSAPESLALAKKLYAEVQRTFPSSRTVHIGGDEWGDDVTAAQRVTWMNAMAAALDDREVWAWNDGIDRVAVGRLDPRIHVTYWSFDGDTEDAAERRERRARRASAVDLQQAGIDQLNYNSYYLYEVPTDLDPADSDYTVADLRENWSLRAWDGDSGSLLAAPMSGAAVAIWGEDLEDPPSDALLRWSAPHVTAMIETAAS

SEQ ID NO: 11 - protein, 445 aa, Curtobacterium luteum
DTAVSAVTVTKVTASTTGTAVRTTLKVENTAPVRKPASSVWLYLSAGTEKYTLGRVAVKALSAGSSTSVTAVRGTPSRAAAGKYWVLACAGAYSAKQCRTSTATVTTKPTKRARPETGVMLDVARAYYPVALIKRYIDLLADDGGRFLHLHLTDDQNVGIESTVLGQTPANADLDHGVYTSRVTHRPFLSAAQARTISEYGAERGVTIVPEIDTPGHMAAAFALLEAQHGTKWVDRIRSGENELDTSAPESLVLAKKLYAEVQRTFPSSRTVHIGGDEWGDDVTAAHRVAWMNEMAATLGNREVWAWNDGIDRVAVGRLDPRIHVTYWSFDGDTEDAAERRERRARRASAVDLQQAGIDQLNYNSYYLYEVPTDLDPADSDYTVADLRENWSLRAWDGDSGSLLAAPMSGAAVAIWGEDLEDPPSDALLRWSAPHVTAMIETAAS

SEQ ID NO: 12 - protein, 458 aa, Curtobacterium oceanosedimentum
IGGSAGTADASGAPRLVVTKVTASSTTTSTRTTVRTTLTVKNTSVARKPAADAWLSLTAGSKRYTLGHVSVQSLAAGASATIHATHTAPPRAPAGKYAVLACTGAFSLSKCGTSATTVTTARATRARPDTGVMLDVARAYYPVALIEQYIALLADHGGRFLHLHLTDDQNVGIESEVLGQTLANADLRDGVYTSRITGRPFLSAAQAREISRYAAQRGIAIIPEIDTPGHMAAAFALLEAGHGKQWVDRIRSGESELDTSAPGSSALAARLLQEVTRTFPSSRTVHIGGDEWGDDVTADERVQWLNTMAAAVGNRAVWAWNDGIDRAAIGRLDPRIHVTYWSFDGDTEDATERRERRERRAGANDLYAAGIDLLNYNSYYLYEVPTDLDAADSEYTVADLRENWSLRTWDGDSGARLAGPTSGAAVAIWGEDLEAPPSDALLRWSAPHVLAMIETAGS

SEQ ID NO: 13 - protein, 450 aa, Curtobacterium leaf154
AGSTTSTVTVTQVTATTTASSTGTAVRTTLKIKNTAAVRKPASSAWLYLSAGTKKYTLGRVAVKALAAGSSTSVTAVRGTPSRATAGEYSVLACAGAYSAKQCRTSTATVTTKPTKRARPETGVMLDVARAYYPVALIKRYIDLLADDGGRFLHLHLTDDQNVGIESTVLGQTLANADLDEGVYTSRVTRRPFLSAAQARTISDYAARRGVAIVPEIDTPGHMTAAFDLLEAQHGTKWVDRIRSGENELDTSTPGSLALAKKLYAEVQRTFPASRTVHIGGDEWGDDVSAAERVAWMNAMAAALGNREVWAWNDGIDRVAVGRLDPRIHVTYWSFDGDTEDAAERRERRARRASAVDLQQAGIDMLNYNSYYLYEVPTDLDPADSEYTVADLRENWSLRTWDGDSGSLLAAPMSGAAVAIWGEDLEDPPSDALLRWSAPHVTAMIETAAS

SEQ ID NO: 14 - protein, 324 aa, Terribacillus saccharophilus
QDQEKGITIDISRKYYSIKTLKAIVDEISANGGDYLQLHFSDNESYAIASEFLGQNSENPNSAYLTKKELLSLIAYSNDRNIMVIPDIDLPAHSKGWLNIMKEKDSGLYTDIVTDYSEDTLDYHNNAVALYTANQLLDEVLDLFYQPKFAGKQRIVLGGDEVPGSGAHQTDFIRFMNQIAKTAKASNYEPQMWNDSITPEGIQNLDRSFSILYWKQSTLSNGAQSLDVQDFEENGLSVYNYNAYSLYFLPSTRFTQEDITEQIDYMKWAYAYNKFFYISDYYKQVDTPNVKGSSLVFWGEHANDLSQEGLLKQEKPLIQNFLGL

SEQ ID NO: 15 - protein, 324 aa, Terribacillus goriensis
QDQEKGITIDISRKYYSIETLKSIIDEISANGGDYLQLHFSDNERYAIASEFLGQNGENPNSTYLTKKELLSLIAYSNDRDIMVIPDIDLPAHSRGWLNIMKEKDSGLYTDIVTDYSEDTLDYHNNAVALYTANQLLDEVLDLFYQPKFAGKQRIVLGGDEVPGSGVHQTDFIRFMNQIAETAKASNYKPQMWNDSITPEGIQNLDRSFSILYWKQSTLSNGAQGLDVQDFEENGLSVYNYNAYSLYFLPATRFTQEDITEQIDYMKWAYAYNKFFYISDYYKQVDTSNVKGSSLVFWGEHANDLSQEGLLKQEKPLIQNFLGL

SEQ ID NO: 16 - protein, 324 aa, Terribacillus saccharophilus
KDQEKGITIDISRKYYSIGTLKAIVDEINANGGDYLQLHFSDNESYAIASEFLGQNSENPNSTYLTKKELLSLIAYSNDRNIMVIPDIDLPAHSKGWLNVMKEKDSGLYTDIVTDYSEDTLDYHNNAAALYTANQLLDEVLDLFYQPKFAGKQRIVLGGDEVPGSGAHQTDFIRFMNQIDETAKASNYEPQMWNDSITPEGIQNLDRSFSILYWKQSTLSSGAQGLDVQNFEEKGFSVYNYNAYSLYFLPSTRFTQEDITEQIDYMKWAYAYNKFFYISDYYKQVDTSNVKGSSLVFWGEHANDLSQEGLLEQEKPLIQNFLSL

SEQ ID NO: 17 - protein, 324 aa, Terribacillus saccharophilus [sequence omitted]

SEQ ID NO: 18 - protein, 324 aa, Terribacillus saccharophilus
KDQEKGISIDISRKYYSIGTLKAIIDEISANGGDYLQLHFSDNESYAIASDYLGQISDTPNNTYLTKNDLLSLIAYSNDRNILIIPDMDLPAHSRGWLELMKVKDRELYTDIVTDYSNETLDYHNNTDALNTANQLLNEILELFYQPKFAGKQRIVLGGDEVPGSEIHQLDFIRFINQIASTAKASNYAPQMWNDSITAEGIQNLDKSFSILYWKQSTLSNGAQSLEVQDFEDWDFPVYNYNAYSLYFLPSIRFTDEDITEQMNYMKWAYAYNKFFYISDYYKSVDASNVKGSSLTFWGEHATDLSQEELLEQELPLIKKFLSL

SEQ ID NO: 19 - protein, 331 aa, Lactobacillus paraplantarum
NSSTLNTSQGVMLDLGRHPLDETAIKAVISAAAEQHMQYVELHLSDNEHLCFQSAYLGNAASATVLSATTLEQLVAYANQLNIELVPDVDLPSHAGAILRQLQQTHPDIYNTVKLDDETIDYTKPAAISLATTLYGELDASFNNQSQHDLMLGADEVPGSASAYIELTTFINQVSRFQNQHGFNTSIWNDSLLKNELTRLDSNITINYWSQSGNNTDVAIIADRYANRVSVPDILASGHPIVNCNSYATYYQIKNIGNVNDDDYFINYLNHTFRPNIFNEIDTNGHNQDWTIEDGVTTNGILVSLWGADSEHVTPTAIVNFIKRMTIPRSF

SEQ ID NO: 20 - protein, 353 aa, Lactobacillus apinorum
TLADTSNDTKRIGLSLDCSRTYYSPSTIKKYIDLLKKDHGTYLQLHLNDNERYGVESSTLGQTTQNATLKDGVYYNNKTHLAFLSKNQLLDVIQYGYTHGIEVIPEIDLPGHAQSIFKLLSYTSEGKKLVKELENKDGYNEMYYNKQATIDFSKKLLSEYVGMLPSGYHIIVGADEITISDKSDQEAVVKYINAIDDYVNANHLKLEMWNDSFHKAVLSKYHKDILINYWSLTGEVSSSKDRKDNIRMRATLPELNKAGFKTINYNSYYLYMITDPTSFTNESKKIWTSEFKKWKMNMWNDESTKDITKSANNIGAAISIWGEYPNQYTGDQTYNKTYYYVDTFLKAQDKFTK

SEQ ID NO: 21 - protein, 331 aa, Lactobacillus paraplantarum
NSSTLNTSQGVMLDLGRHPLDETAIKAVISAAAEQHMQYVELHLSDNEHLCFQSAYLGNAASATVLSATTLEQLVAYANQLNIELVPDVDLPSHAGAILRQLQQTHPDIYNTVKLDDETIDYTKPAAVSLATTLYGELDASFNNQSQHDLMLGADEVSGSASAYIELTTFINQVSRFQNQNGFNTSIWNDSLLKNELNRLDSNITINYWSQSGNNTDAAIIADRYANRASVPDILASGHPIVNCNSYATYYQFKNIGNVNDDNYFINYLNHTFRPNIFNEIDTNGHNQDWTIEDGVTTNGILVSLWGADSEHVTPTAIVNFIKRMAIPRSF

SEQ ID NO: 22 - protein, 323 aa, Staphylococcus cohnii
QDFQKGINVDIARKDYSLKSLKKIVDTIHENNGDYLQLHFSDNENYAIESQFFKHENIASQNYLSQQELKNLIHYSNKLNIMVVPEFDLPSHSKAWLLLLKNENSNLHENIVSDYSDETIDFFSNQKALEISKRQIKEILNLFHQPNFQKEQRIVLGGDEVPGGKSYQNDFINFMNEIGEYAYQNGYEPQIWNDSITKNGLKLLKNYFSVIFWKQSNNENNEPGITVEDFLDYNFKVYNYNFYSLYFLPSKNYSPTDIEEQTSYISWAYNHNSFYYLKNPYYEVDSLNIQGSALSFWGEHATGMREEEVLNQELPLIRTYLNK

SEQ ID NO: 23 - protein, 321 aa, Staphylococcus fleurettii
ESIQEGVSVDIARKEYSLESLKQIVDTIHENNGQYLQLHFSDDENYAIESDYFSHQGIPNENYLTKAEIKSLIAYSNELNVMVVPDIDFPSHSKALLSLIKNEDKDLYNQIISDYSDNTFDFFSNDKALAISKRHIGEITTLFNQPKYNGQQRIVLGGDEVPGGGAYQSDFISYMNNIGSYAAGQGYEPQMWNDMISHEGIKSLNDTFSILYWKQNENSKSDLTVEDFAEYDFKIYNYNFYSLYFLPSNQFTNADIEEQADYISWAYAYNKFFYTNEPYQEVDSDNVKGSALSFWGEDALNMSQTELINQEIPLIKAYFSS

SEQ ID NO: 24 - protein, 298 aa, Bacillus bogoriensis
ANSGFYVSGTTLYDANGNPFVMRGINHGHAWYKDQATTAIEGIANTGANTVRIVLSDGGQWTKDDIHTVRNLISLAEDNHLVAVLEVHDATGYDSIASLNRAVDYWIEMRSALIGKEDTVIINIANEWFGSWEGDAWADGYKQAIPRLRNAGLNHTLMVDAAGWGQFPQSIHDYGREVFNADPQRNTMFSIHMYEYAGGNASQVRTNIDRVLNQDLALVIGEFGHRHTNGDVDEATIMSYSEQRGVGWLAWSWKGNGPEWEYLDLSNDWAGNNLTAWGNTIVNGPYGLRETSRLSTVF

SEQ ID NO: 25 - protein, 278 aa, thielavia terrestris
ASGSGQSTRYWDCCKPSCAWPGKAAVSQPVYACDANFQRLSDFNVQSGCNGGSAYSCADQTPWAVNDNLAYGFAATSIAGGSESSWCCACYALTFTSGPVAGKTMVVQSTSTGGDLGSNQFDIAMPGGGVGIFNGCSSQFGGLPGAQYGGISSRDQCDSFPAPLKPGCQWRFDWFQNADNPTFTFQQVQCPAEIVARSGCKRNDDSSFPVFTPPSGGNGGTGTPTSTAPGSGQTSPGGGSGCTSQKWAQCGGIGFSGCTTCVSGTTCQKLNDYFSQCL

SEQ ID NO: 26 - protein, 470 aa, humicola insolens
MRSSPLLRSAVVAALPVLALAADGRSTRYWDCCKPSCGWAKKAPVNQPVFSCNANFQRITDFDAKSGCEPGGVAYSCADQTPWAVNDDFALGFAATSIAGSNEAGWCCACYELTFTSGPVAGKKMVVQSTSTGGDLGSNHFDLNIPGGGVGIFDGCTPQFGGLPGQRYGGISSRNECDRFPDALKPGCYWRFDWFKNADNPSFSFRQVQCPAELVARTGCRRNDDGNFPAVQIPSSSTSSPVNQPTSTSTTSTSTTSSPPVQPTTPSGCADGRSTRYWDCCKPSCGWAKKAPVNQPVFSCNANFQRITDFDAKSGCEPGGVAYSCADQTPWAVNDDFALGFAATSIAGSNEAGWCCACYELTFTSGPVAGKKMVVQSTSTGGDLGSNHFDLNIPGGGVGIFDGCTPQFGGLPGQRYGGISSRNECDRFPDALKPGCYWRFDWFKNADNPSFSFRQVQCPAELVARTGCRR

SEQ ID NO: 27 - protein, 425 aa, Escherichia coli
TALLLGLVNGQKPGETKEVHPQLTTFRCTKRGGCKPATNFIVLDSLSHPIHRAEGLGPGGCGDWGNPPPKDVCPDVESCAKNCIMEGIPDYSQYGVTTNGTSLRLQHILPDGRVPSPRVYLLDKTKRRYEMLHLTGFEFTFDVDATKLPCGMNSALYLSEMHPTGAKSKYNPGGAYYGTGYCDAQCFVTPFINGLGNIEGKGSCCNEMDIWEANSRASHVAPHTCNKKGLYLCEGEECAFEGVCDKNGCGWNNYRVNVTDYYGRGEEFKVNTLKPFTVVTQFLANRRGKLEKIHRFYVQDGKVIESFYTNKEGVPYTNMIDDEFCEATGSRKYMELGATQGMGEALTRGMVLAMSIWWDQGGNMEWLDHGEAGPCAKGEGAPSNIVQVEPFPEVTYTNLRWGEIGSTYQEVQKPKPKPGHGPRSD

SEQ ID NO: 28 - protein, 773 aa, bacillus subtilis
AEGNTREDNFKHLLGNDNVKRPSEAGALQLQEVDGQMTLVDQHGEKIQLRGMSTHGLQWFPEILNDNAYKALANDWESNMIRLAMYVGENGYASNPELIKSRVIKGIDLAIENDMYVIVDWHVHAPGDPRDPVYAGAEDFFRDIAALYPNNPHIIYELANEPSSNNNGGAGIPNNEEGWNAVKEYADPIVEMLRDSGNADDNIIIVGSPNWSQRPDLAADNPINDHHTMYTVHFYTGSHAASTESYPPETPNSERGNVMSNTRYALENGVAVFATEWGTSQANGDGGPYFDEADVWIEFLNENNISWANWSLTNKNEVSGAFTPFELGKSNATNLDPGPDHVWAPEELSLSGEYVRARIKGVNYEPIDRTKYTKVLWDFNDGTKQGFGVNSDSPNKELIAVDNENNTLKVSGLDVSNDVSDGNFWANARLSADGWGKSVDILGAEKLTMDVIVDEPTTVAIAAIPQSSKSGWANPERAVRVNAEDFVQQTDGKYKAGLTITGEDAPNLKNIAFHEEDNNMNNIILFVGTDAADVIYLDNIKVIGTEVEIPVVHDPKGEAVLPSVFEDGTRQGWDWAGESGVKTALTIEEANGSNALSWEFGYPEVKPSDNWATAPRLDFWKSDLVRGENDYVAFDFYLDPVRATEGAMNINLVFQPPTNGYWVQAPKTYTINFDELEEANQVNGLYHYEVKINVRDITNIQDDTLLRNMMIIFADVESDFAGRVFVDNVRFEGAATTEPVEPEPVDPGEETPPVDEKEAKKEQKEAEKEEKEE

SEQ ID NO: 29 - protein, 524 aa, Paenibacillus polymyxa
VVHGQTAKTITIKVDTFKDRKPISPYIYGTNQDLAGDENMAARRLGGNRMTGYNWENNMSNAGSDWQHSSDNYLCSNGGLTQAECEKPGAVVTSFHDQSLKLGTYSLVTLPMAGYVAADGNGSVQESEAAPSARWNQVVNAKNAPFQLQPDLNDNYVYVDEFVHFLVNKYGTASTKAGVKGYALDNEPALWSHTHPRIHPEKVGAKELVDRSVSLSKAVKAIDAGAEVFGPVLYGFGAYKDLQTAPDWDSVKGNYSWFVDYYLDQMRLSSQVEGKRLLDVFDVHWYPEAMGGGIRITNEVGNDETKKARMQAPRTLWDPTYKEDSWIAQWFSEFLPILPRLKQSVDKYYPGTKLAMTEYSYGGENDISGGIAMTDVLGILGKNDVYMANYWKLKDGVNNYVSAAYKLYRNYDGKNSTFGDTSVSAQTSDIVNSSVHASVTNASDKELHLVVMNKSMDSAFDAQFDLSGAKTYISGKVWGFDKNSSQIKEAAPITQISGNRFTYTVPPLTAYHIVLTTGNDTSPV

SEQ ID NO: 30 - protein, 485 aa, Bacillus sp.
HHNGTNGTMMQYFEWYLPNDGNHWNRLRSDASNLKDKGISAVWIPPAWKGASQNDVGYGAYDLYDLGEFNQKGTIRTKYGTRNQLQAAVNALKSNGIQVYGDVVMNHKGGADATEMVRAVEVNPNNRNQEVSGEYTIEAWTKFDFPGRGNTHSNFKWRWYHFDGVDWDQSRKLNNRIYKFRGDGKGWDWEVDTENGNYDYLMYADIDMDHPEVVNELRNWGVWYTNTLGLDGFRIDAVKHIKYSFTRDWINHVRSATGKNMFAVAEFWKNDLGAIENYLNKTNWNHSVFDVPLHYNLYNASKSGGNYDMRQIFNGTVVQRHPMHAVTFVDNHDSQPEEALESFVEEWFKPLAYALTLTREQGYPSVFYGDYYGIPTHGVPAMKSKIDPILEARQKYAYGRQNDYLDHHNIIGWTREGNTAHPNSGLATIMSDGAGGNKWMFVGRNKAGQVWTDITGNRAGTVTINADGWGNFSVNGGSVSIWVNK

SEQ ID NO: 31 - protein, 485 aa, Bacillus sp. NCIB 12513
HHNGTNGTMMQYFEWHLPNDGNHWNRLRDDASNLRNRGITAIWIPPAWKGTSQNDVGYGAYDLYDLGEFNQKGTVRTKYGTRSQLESAIHALKNNGVQVYGDVVMNHKGGADATENVLAVEVNPNNRNQEISGDYTIEAWTKFDFPGRGNTYSDFKWRWYHFDGVDWDQSRQFQNRIYKFRGDGKAWDWEVDSENGNYDYLMYADVDMDHPEVVNELRRWGEWYTNTLNLDGFRIDAVKHIKYSFTRDWLTHVRNATGKEMFAVAEFWKNDLGALENYLNKTNWNHSVFDVPLHYNLYNASNSGGNYDMAKLLNGTVVQKHPMHAVTFVDNHDSQPGESLESFVQEWFKPLAYALILTREQGYPSVFYGDYYGIPTHSVPAMKAKIDPILEARQNFAYGTQHDYFDHHNIIGWTREGNTTHPNSGLATIMSDGPGGEKWMYVGQNKAGQVWHDITGNKPGTVTINADGWANFSVNGGSVSIWVKR

SEQ ID NO: 32 - protein, 485 aa, Bacillus sp. no. 707
HHNGTNGTMMQYFEWYLPNDGNHWNRLNSDASNLKSKGITAVWIPPAWKGASQNDVGYGAYDLYDLGEFNQKGTVRTKYGTRSQLQAAVTSLKNNGIQVYGDVVMNHKGGADATEMVRAVEVNPNNRNQEVTGEYTIEAWTRFDFPGRGNTHSSFKWRWYHFDGVDWDQSRRLNNRIYKFRGHGKAWDWEVDTENGNYDYLMYADIDMDHPEVVNELRNWGVWYTNTLGLDGFRIDAVKHIKYSFTRDWINHVRSATGKNMFAVAEFWKNDLGAIENYLQKTNWNHSVFDVPLHYNLYNASKSGGNYDMRNIFNGTVVQRHPSHAVTFVDNHDSQPEEALESFVEEWFKPLAYALTLTREQGYPSVFYGDYYGIPTHGVPAMRSKIDPILEARQKYAYGKQNDYLDHHNILGWTREGNTAHPNSGLATIMSDGAGGSKWMFVGRNKAGQVWSDITGNRTGTVTINADGWGNFSVNGGSVSIWVNK

SEQ ID NO: 33 - protein, 485 aa, Artificial
  fusion protein
HHDGTNGTIMQYFEWNVPNDGQHWNRLHNNAQNLKNAGITAIWIPPAWKGTSQNDVGYGAYDLYDLGEFNQKGTVRTKYGTKAELERAIRSLKANGIQVYGDVVMNHKGGADFTERVQAVEVNPQNRNQEVSGTYQIEAWTGFNFPGRGNQHSSFKWRWYHFDGTDWDQSRQLANRIYKFRGDGKAWDWEVDTENGNYDYLMYADVDMDHPEVINELNRWGVWYANTLNLDGFRLDAVKHIKFSFMRDWLGHVRGQTGKNLFAVAEYWKNDLGALENYLSKTNWTMSAFDVPLHYNLYQASNSSGNYDMRNLLNGTLVQRHPSHAVTFVDNHDTQPGEALESFVQGWFKPLAYATILTREQGYPQVFYGDYYGIPSDGVPSYRQQIDPLLKARQQYAYGTQHDYLDNQDVIGWTREGDSAHAGSGLATVMSDGPGGSKTMYVGTAHAGQVFKDITGNRTDTVTINSAGNGTFPCNGGSVSIWVKQ

SEQ ID NO: 34 - protein, 330 aa, Paenibacillus woosongensis
IRTGTLNNPEATAEARALMNYLLSQYGQKIISGQQTLEDVEWIKQQTGKYPAIFSTDLMDYSPSRVDHGASSTEVEKMIEWYKRGGIVSLCWHWNAPKGIGGNEPGNEWWRGFYTEFTTFDVEYALNHPDSEDYQLLIRDIDAIAVQLKRLQEANVPVLWRPLHEAEGTWFWWGAKGPEPAKQLYRLMYDRLTNDHKLNNLIWVWNSEKKDWYPGDDVVDMVSVDIYNPAGDYNPSIAKYEALVSLADNKKMAALAENGPIPDPDALQEYGADWSFFSTWTGDYIRDGKTNTIEHLKKVYQHDYVITLDELPADCTPILMIRQRMVNQQG

SEQ ID NO: 35 - protein, 312 aa, Paenibacillus illinoisensis
ASPQAKALMKFMTNQYGKKIISGQQTLEDAAWIYQQTGKYPALVSSDLMDYSPSRVENGSTSNEVEKMMEWYKRGGIVSLSWHWNAPKGIGSNEPGHEWWRGFNTEFTTFDVEYALNHPESEDYKLLIRDIDAIATQLKRLQEHHIPVLWRPLHEAEGGWFWWGAKGPEPAKKLYRLMYERLTEKHGLNNLIWVWNSVKEEWYPGDDVVDMVSVDIYNPPGDYSPNIAKYDELLFLSKHKKLVALAENGPIPDPDLLQTYGAHWSYFNTWTGDVLRDGKTNTKEHLKKVYNHDNVITLDELPKGLYDSPRWK

SEQ ID NO: 36 - protein, 699 aa, Neobulgaria sp.
TVFEAEKGTLAGGLTIATDVTGYTGTGYVTNFADAAALLTFTVNGLTAGSYDLTLTYSAQYGDKFTTVSVNGASGIEVAITNVTTATWTTATIGTFTLTAGDNTVSCADDWGWYLIDSLTVIPTPAKPITIVDVSNGATAQAEDGILTGTTVGTTTAGYTGTGYVTGFTATGTQVTINLSSTKQALYDVVVRYAAIYGQKYTTMQLNGVGGSEILLLDTTTATSPWANATAGQVLLASGNNTLTFMNDWGWYFIDAVYVTPSPAPAPHKVTNALVDAKALASTHALFNTLLAKYGSGDIFSGQADPTGVTWIESNLGTTKTPAIIGLDMIEYSPTRVLYGSTSTAVEDAIAFDKRGGMVAFQWHWNAPADLINNDTVPWWKGFYSYGTTFNLTAALANPSGSDYALLISDMDAIAVQLLRLQAAGVPVLWRPLHEADGTWFWWGNFGAASCVSLYRIMYDRYTNYHGLHNLIWVWNSVTPSWYPGADVVDILGYDSYPAVGDHGPVSSQYNALITLGGDTKLVTLPEVGNIPDPAILKLYHADWSYFVTWNQDYILTDTYNPLAFKQQVYNDPTVLKLTDLGNWKGAATSTIVSSTSKVSTTTSSLITSTTKKTSSSTVVSTTSSTVKTTSTTSKVSSSTTKVSSTTKVTTTSTTTSAVATATAGHWGQCGGTGWTGPTVCASGFTCTAVSPPYYYQCL

SEQ ID NO: 37 - protein, 452 aa, Preussia aemulans
QTVIYQAEQAKLSGVTVEFSIIKQVVGTGYVEGFDESTDSITFTVESTTAALYDLALTYNGPYGDKYTNVVLNNAAGSQVSLPATTAWTTVPAGQVLLNAGANTIQIQNNWGWYLVDSISLKPAATRGAHQITTKPVNKNANSDAKALLKYLGSIYGKKILSGQQDLSSLDWVTKNVGKTPAVLGLDTMDYSESRKSRGAVSTDVDKAIAFAKKGGIVTFCWHWGAPTGLFDSAAQPWYRGFYTDATDFNIETALKDTTNANYTLLMKDIDTIAVQLKKLQDAGVPVIWRPLHEAEGGWFWWGAKGPEPAKKLWKIMYDRLTNQHGLNNLVWTWNSVAPNWYPGDDTVDIVSADTYSQGDHGPISATYNNLLALTNDTKIIAAAEIGSVMEPAQLQAYQADWVYFCVWSGEFIDGGVWNSLDFLKKVYNDPYVLTLDEIQGWKTARGKPRVS

SEQ ID NO: 38 - protein, 312 aa, Yunnania penicillata
APSTTPVNEKATDAAKNLLSYLVEQAANGVTLSGQQDLESAQWVSDNVGKWPAILGIDFMDYSPSRVEYGAVGSTVPDAISYDSDGGIVTFCWHWGSPSGTYNTTDQPWWSNFYTEATAFDIAAAMDDPDSADYNLLVRDIDAISELLLQLQDLDIPILWRPLHEAEGGWFWWGAKGPEACIALYRLMFDRMTNHHGLNNLLWVWNSVDPSWYPGNDVVDIVSADIYADAGDHSPQEETFASLQSLTGDTKLVALGEVGNIPDPASTGGVADWAYWVTWNGDFIKGEDYNPLEYKKEVFSAENIITRDEVDV

SEQ ID NO: 39 - protein, 327 aa, Myrothecium roridum
GTIENRQWLTYNPVDSAATTEARALLRYIQSQYGWRYLSGQQERAEVQWLKSNIGKTPAIQGSDLIDYSPSRVSYGATSTAVEDAIAFDRQGGIVTFTWHWNAPNCLYNSADQPWYFGFYTKATCFNIQAALAQGSNGADYKLLIRDIDAIAVQLKRLRDAKVPILFRPLHEPDGAWFWWGAKGSGPFKQLWDILYDRLTKYHGLHNMLWVCNTEKSDWYPGNNKCDIATTDVYVNAGDHSVQKSHWDALYGVSGGQRILALGEVGVIPDPERQASENVPWAYWMTWNGYFIRDGNYNSRNFLQSTFSNARVVTLDGTSPLGNWKSS

SEQ ID NO: 40 - protein, 452 aa, Chaetomium brasiliense
VPCGGGSNSGPRTYEAEDADLTGTNIDTAQSGFTGSGYVTGFDQATDKVTFKVDSPSLKLYDLSIRVAAIYGEKRTNVVLNNGASSEVYFAASETFTTVAAGQVLLNEGANTIDLVSNWGWYLIDSITLTPSTQRPPHNINPSPVNPSANADAKGLYTYLRSIYGKKILSGQQELSWSNWITTQTGKTPALVSVDLMDYSPSRVERGTVGTAVEEAITHAQRGGIVSVLWHWNAPTGLYDTEENKWWSGFYTRATDFDVAAALSSTTNANYTLILRDIDAIAVQLKKLQDAGVPVLFRPLHEAEGGWFWWGAKGAEPCKKLYALLYDRLTNYHKINNLIWVWNSILEEWYPGDATVDILSADVYAQGNGPISTQYNQLIELGKDKKMIAAAEVGAAPLPNLLQAYEAHWLWFTVWGDTFINNAEWNSVDVLKQVYTSDYVLTLDEIQGWRGA

SEQ ID NO: 41 - protein, 541 aa, Ascobolus stictoideus
QTYTLEAEAGTLTGVTVMNEIAGFSGTGYVGGWDEDADTVSLTFTSDATKLYDVKIRYSGPYGSKYTRISYNGATGGDISLPETTEWATVNAGQALLNAGSNTIKLHNNWGWYLIDAVILTPSVPRPPHQVTDALVNTNSNAVTKQLMKFLVSKYHKAYITGQQELHAHQWVEKNVGKSPAILGLDFMDYSPSRVEFGTTSQAVEQAIDFDKRGGIVTFAWHWNAPSGLINTPGSEWWRGFYTEHTTFDVAAALQNTTNANYNLLIRDIDAIAVQLKRLQTAGVPVLWRPLHEAEGGWFWWGAKGPEPAKKLYKILYDRLTNYHKLNNLIWVWNSVAKDWYPGDEIVDVLSFDSYPAQPGDHGPVSAQYNALVELGKDKKLIAATEVGTIPDPDLMQLYESYWSFFVTWEGEFIENGVHNSLEFLKKLYNNSFVLNLDTIQGWKNGAGSSTTTVKSTTTTPTTTIKSTTTTPVTTPTTVKTTTTPTTTATTVKSTTTTAGPTPTAVAGRWQQCGGIGFTGPTTCEAGTTCNVLNPYYSQCL

SEQ ID NO: 42 - protein, 526 aa, Chaetomium virescens
PRDPGATARTFEAEDATLAGTNVDTALSGFTGTGYVTGFDQAADKVTFTVDSASTELYDLSIRVAAIYGDKRTSVVLNGGASSEVYFPAGETWTNVAAGQLLLNQGSNTIDIVSNWGWYLIDSITLTPSTPRPAHQINEAPVNAAADKNAKALYSYLRSIYGKKILSGQQELSLSNWIAQQTGKTPALVSVDLMDYSPSRVERGTVGTAVEEAIQHHNRGGIVSVLWHWNAPTGLYDTEEHRWWSGFYTSATDFDVAAALSSTTNANYTLLIRDIDAIAVQLKRLQSAGVPVLFRPLHEAEGGWFWWGAKGPEPAKKLWGILYDRVTNHHQINNLLWVWNSILPEWYPGDATVDILSADVYAQGNGPMSTQYNQLIELGKDKKMIAAAEVGAAPLPDLLQAYEAHWLWFTVWGDSFINNADWNSLDTLKKVYTSDYVLTLDEIQGWQGSTPSATTTSSTTTPSATTTTTTPSTTATTATPSATTTASPVTYAEHWGQCAGKGWTGPTTCRPPYTCKYQNDWYSQCL

SEQ ID NO: 43 - protein, 483 aa, Cytophaga sp.
AATNGTMMQYFEWYVPNDGQQWNRLRTDAPYLSSVGINAVWTPPAYKGTSQADVGYGPYDLYDLGEFNQKGTVRTKYGTKGELKSAVNTLHSNGIQVYGDVVMNHKAGADYTENVTAVEVNPSNRYQEISGEYNIQAWTGFNFPGRGTTYSNWKWQWFHFDGTDWDQSRSLSRIFKFDGKAWDWPVSSENGNYDYLMYADYDYDHPDVVNEMKKWGVWYANEVGLDGYRLDAVKHIKFSFLKDWVDNARAATGKEMFTVGEYWQNDLGALNNYLAKVNYNQSLFDAPLHYNFYAASTGGGYYDMRNILNNTLVASNPTKAVTLVENHDTQPGQSLESTVQPWFKPLAYAFILTRSGGYPSVFYGDMYGTKGTTTREIPALKSKIEPLLKARKDYAYGTQRDYIDNPDVIGWTREGDSTKAKSGLATVITDGPGGSKRMYVGTSNAGEIWYDLTGNRTDKITIGSDGYATFPVNKESVSVWVQQ